European Patent Application EP 4 520 767 A1, published March 12, 2025. Title: PEPTIDE KINASE INHIBITORS AND METHODS OF USE THEREOF. Applicant: B.G. NEGEV TECHNOLOGIES AND APPLICATIONS LTD. Application US. The sequence listing filed with the application follows.

SEQUENCE LISTING (38 sequences)

SEQ ID NO: 1 - protein, 26 aa, Homo sapiens
MASRGALRRCLSPGLPRLLHLSRGLA

SEQ ID NO: 2 - protein, 33 aa, synthetic construct
  REGION 1..33: note = synthetic polypeptide
MASRGALRRCLSPGLPRLLHLSRGLARRMKWKK

SEQ ID NO: 3 - protein, 17 aa, Homo sapiens
MASRGALRRCLSPGLPR

SEQ ID NO: 4 - protein, 17 aa, synthetic construct
  REGION 1..17: note = synthetic polypeptide
MASRGALRRALSPGLPR

SEQ ID NO: 5 - protein, 26 aa, synthetic construct
  REGION 1..26: note = synthetic polypeptide
MASRGALRRALSPGLPRLLHLSRGLA

SEQ ID NO: 6 - protein, 17 aa, synthetic construct
  REGION 1..17: note = synthetic polypeptide
MASRGSLRRCLSPGLPR

SEQ ID NO: 7 - protein, 17 aa, synthetic construct
  REGION 1..17: note = synthetic polypeptide
MASRGTLRRCLSPGLPR

SEQ ID NO: 8 - protein, 26 aa, synthetic construct
  REGION 1..26: note = synthetic polypeptide
MASRGSLRRCLSPGLPRLLHLSRGLA

SEQ ID NO: 9 - protein, 26 aa, synthetic construct
  REGION 1..26: note = synthetic polypeptide
MASRGTLRRCLSPGLPRLLHLSRGLA

SEQ ID NO: 10 - protein, 7 aa, synthetic construct
  REGION 1..7: note = synthetic polypeptide
RRMKWKK

SEQ ID NO: 11 - protein, 18 aa, Homo sapiens
MGPREARLQVHQLQTAGP

SEQ ID NO: 12 - protein, 16 aa, synthetic construct
  REGION 1..16: note = synthetic polypeptide
MGPREARLQVHQLQTA

SEQ ID NO: 13 - skipped

SEQ ID NO: 14 - protein, 5 aa, Homo sapiens
KKKRR

SEQ ID NO: 15 - protein, 7 aa, Homo sapiens
PKKKRRV

SEQ ID NO: 16 - protein, 8 aa, Homo sapiens
KRRMKWKK

SEQ ID NO: 17 - protein, 5 aa, Homo sapiens
KKKRK

SEQ ID NO: 18 - protein, 5 aa, Homo sapiens
KKKRK

SEQ ID NO: 19 - protein, 17 aa, Homo sapiens
TRKRQRAMRRRVHHQIN

SEQ ID NO: 20 - protein, 26 aa, Macaca mulatta
MASRGALGRCLSPGLPRLLQLSRGLA

SEQ ID NO: 21 - protein, 26 aa, Elephas maximus
MAGRGGLGRCFSPELPPLLRLPRGLA

SEQ ID NO: 22 - protein, 26 aa, Canis familiaris
MTSGGGLGRCFSPELRPLRRLPRGLA

SEQ ID NO: 23 - protein, 26 aa, Mus musculus
MAGRRGLGRCFFPELPPRPWQRRGLP

SEQ ID NO: 24 - protein, 26 aa, Rattus rattus
MAGRRGLGCCFSRELPPRAWLRRGLP

SEQ ID NO: 25 - protein, 18 aa, Homo sapiens
RFARKGALRQKNVHEVKD

SEQ ID NO: 26 - protein, 18 aa, Homo sapiens
RFARKGALRQKNVHEVKN

SEQ ID NO: 27 - protein, 18 aa, Homo sapiens
LFCRKGALRQKVVHEVKS

SEQ ID NO: 28 - protein, 18 aa, Homo sapiens
TMNRRGAIKQAKIHYIKN

SEQ ID NO: 29 - protein, 17 aa, Homo sapiens
PRKRQGAVRRRVHHQVN

SEQ ID NO: 30 - protein, 17 aa, Homo sapiens
SIYRRGARRWRKLYRAN

SEQ ID NO: 31 - protein, 17 aa, Homo sapiens
HQRRGAIKQAKVHHVKC

SEQ ID NO: 32 - protein, 26 aa, synthetic construct
  REGION 1..26: note = Synthetic polypeptide
  SITE 10: note = MISC_FEATURE - X is C or A
MASRGALRRXLSPGLPRLLHLSRGLA

SEQ ID NO: 33 - DNA, 61 bp, synthetic construct
  misc_feature 1..61: note = synthetic polynucleotide
  source 1..61: mol_type = other DNA
gatccccggcccgtcttaactccgattgatctcgatcaatcggagttaagacgggtttttg

SEQ ID NO: 34 - DNA, 75 bp, synthetic construct
  misc_feature 1..75: note = synthetic polynucleotide
  source 1..75: mol_type = other DNA
gatccccgggggtctccaacccggaaatatctccttcctgtcagagagatatttccgggttggagaccctttttg

SEQ ID NO: 35 - DNA, 69 bp, synthetic construct
  misc_feature 1..69: note = synthetic polynucleotide
  source 1..69: mol_type = other DNA
gatccccggccatcaagtgaacggacataacttcctgtcagattatgtccgttcacttgatggtttttg

SEQ ID NO: 36 - protein, 26 aa, synthetic construct
MASRGALARCLSPGLPRLLHLSRGLA

SEQ ID NO: 37 - protein, 26 aa, synthetic construct
MASRGALARALSPGLPRLLHLSRGLA

SEQ ID NO: 38 - protein, 26 aa, synthetic construct
MASRGALRRCLAPGLPRLLHLSRGLA